European Patent Specification EP 3 377 653 B1, published October 29, 2025. Title: METHODS FOR OBTAINING AND CORRECTING BIOLOGICAL SEQUENCE INFORMATION. Applicant: Cygnus Biosciences (Beijing) Co., Ltd. Application Not Yet Assigned. The sequence listing filed with the application follows.

SEQUENCE LISTING (41 sequences)

SEQ ID NO: 1 - DNA, 15 bp, Artificial Sequence
  Synthetic
aactttggattgcct

SEQ ID NO: 2 - DNA, 20 bp, Artificial Sequence
  Synthetic
tgaactttagccacggagta

SEQ ID NO: 3 - DNA, 31 bp, Artificial Sequence
  Synthetic
  PS3-T10-P7
ttttttttttcaagcagaagacggcatacga

SEQ ID NO: 4 - DNA, 20 bp, Artificial Sequence
  Synthetic
  P5
aatgatacggcgaccaccga

SEQ ID NO: 5 - DNA, 21 bp, Artificial Sequence
  Synthetic
  P7
caagcagaagacggcatacga

SEQ ID NO: 6 - DNA, 58 bp, Artificial Sequence
  Synthetic
  P5-SeqP1
aatgatacggcgaccaccgagatctacactctttccctacacgacgctcttccgatct

SEQ ID NO: 7 - DNA, 21 bp, Artificial Sequence
  Synthetic
  FAM-P7rc
tcgtatgccgtcttctgcttg

SEQ ID NO: 8 - DNA, 35 bp, Artificial Sequence
  Synthetic
  FAM-T-SeqP1
ttacactctttccctacacgacgctcttccgatct

SEQ ID NO: 9 - DNA, 55 bp, Artificial Sequence
  Synthetic
  Adp1-L10115-301-f
acactctttccctacacgacgctcttccgatctgtgttcgacggtgagctgagtt

SEQ ID NO: 10 - DNA, 54 bp, Artificial Sequence
  Synthetic
  Adp2-L10115-301-r
gtgactggagttcagacgtgtgctcttccgatctcaagccctgccgctttctgc

SEQ ID NO: 11 - DNA, 55 bp, Artificial Sequence
  Synthetic
  Adp1-L4418-305-f
acactctttccctacacgacgctcttccgatctgtgacagcagagctgcgtaatc

SEQ ID NO: 12 - DNA, 54 bp, Artificial Sequence
  Synthetic
  Adp2-L4418-305-r
gtgactggagttcagacgtgtcatgcgatcatatgagtacggctgcagcgcccg

SEQ ID NO: 13 - DNA, 57 bp, Artificial Sequence
  Synthetic
  Adp1-L718-308-f
acactctttccctacacgacgctcttccgatcttatcgaacagtcaggttaacaggc

SEQ ID NO: 14 - DNA, 54 bp, Artificial Sequence
  Synthetic
  Adp2-L718-308-r
gtgactggagttcagacgtgtcatgcgatcatatcaaccagataagggtgttgc

SEQ ID NO: 15 - DNA, 53 bp, Artificial Sequence
  Synthetic
  Adp1-L501-500-f
acactctttccctacacgacgctcttccgatctactccgctgaagtggtggaa

SEQ ID NO: 16 - DNA, 54 bp, Artificial Sequence
  Synthetic
  Adp2-L501-500-r
gtgactggagttcagacgtgtcatgcgatcatatttatgctctataaagtaggc

SEQ ID NO: 17 - DNA, 53 bp, Artificial Sequence
  Synthetic
  Adp1-L30501-500-f
acactctttccctacacgacgctcttccgatctcactcacaacaatgagtggc

SEQ ID NO: 18 - DNA, 54 bp, Artificial Sequence
  Synthetic
  Adp2-L30501-500-r
gtgactggagttcagacgtgtcatgcgatcatatcacggaatgcatttttctgg

SEQ ID NO: 19 - DNA, 53 bp, Artificial Sequence
  Synthetic
  Adp1-L46499-500-f
acactctttccctacacgacgctcttccgatctgcctaaagtaataaaaccga

SEQ ID NO: 20 - DNA, 54 bp, Artificial Sequence
  Synthetic
  Adp2-L46499-500-r
gtgactggagttcagacgtgtcatgcgatcatatggcataatgcaatacgtgta

SEQ ID NO: 21 - DNA, 53 bp, Artificial Sequence
  Synthetic
  Adp1-L8703-1012-f
acactctttccctacacgacgctcttccgatctaagagctggacagcgatacc

SEQ ID NO: 22 - DNA, 54 bp, Artificial Sequence
  Synthetic
  Adp2-L8703-1012-r
gtgactggagttcagacgtgtgctcttccgatctcatcgctgactctccggatt

SEQ ID NO: 23 - DNA, 57 bp, Artificial Sequence; identical to SEQ ID NO: 13
  Synthetic
  Adp1-L718-208-f

SEQ ID NO: 24 - DNA, 54 bp, Artificial Sequence
  Synthetic
  Adp2-L718-208-r
gtgactggagttcagacgtgtgctcttccgatcttcgctgcccatcgcattcat

SEQ ID NO: 25 - DNA, 55 bp, Artificial Sequence; identical to SEQ ID NO: 9
  Synthetic
  Adp1-L10115-201-f

SEQ ID NO: 26 - DNA, 54 bp, Artificial Sequence
  Synthetic
  Adp2-L10115-201-r
gtgactggagttcagacgtgtgctcttccgatctgctgaaaaacaggctgagca

SEQ ID NO: 27 - DNA, 51 bp, Artificial Sequence
  Synthetic
  P7-Adp2-r
caagcagaagacggcatacgagatactgacgtgactggagttcagacgtgt

SEQ ID NO: 28 - DNA, 45 bp, Artificial Sequence
  Synthetic
  P5-Adp1-f
aatgatacggcgaccaccgagatctacactctttccctacacgac

SEQ ID NO: 29 - DNA, 201 bp, Artificial Sequence
  Synthetic
  L10115-201
gtgttcgacggtgagctgagttttgccctgaaactggcgcgtgagatggggcgacccgactggcgtgccatgcttgccgggatgtcatccacggagtatgccgactggcaccgcttttacagtacccattattttcatgatgttctgctggatatgcacttttccgggctgacgtacaccgtgctcagcctgtttttcagc

SEQ ID NO: 30 - DNA, 193 bp, Artificial Sequence
  Synthetic
  L718-208
tatcgaacagtcaggttaacaggctgcggcattttgtccgcgccgggcttcgctcactgttcaggccggagccacagaccgccgttgaatgggcggatgctaattactatctcccgaaagaatccgcataccaggaagggcgctgggaaacactgccctttcagcgggccatcatgaatgcgatgggcagcga

SEQ ID NO: 31 - DNA, 308 bp, Artificial Sequence
  Synthetic
  L10115-301
tatcgaacagtcaggttaacaggctgcggcattttgtccgcgccgggcttcgctcactgttcaggccggagccacagaccgccgttgaatgggcggatgctaattactatctcccgaaagaatccgcataccaggaagggcgctgggaaacactgccctttcagcgggccatcatgaatgcgatgggcagcgactacatccgtgaggtgaatgtggtgaagtctgcccgtgtcggttattccaaaatgctgctgggtgtttatgcctactttatagagcataagcagcgcaacacccttatctggttg

SEQ ID NO: 32 - DNA, 305 bp, Artificial Sequence
  Synthetic
  L4418-305
gtgacagcagagctgcgtaatctcccgcatattgccagcatggcctttaatgagccgctgatgcttgaacccgcctatgcgcgggttttcttttgtgcgcttgcaggccagcttgggatcagcagcctgacggatgcggtgtccggcgacagcctgactgcccaggaggcactcgcgacgctggcattatccggtgatgatgacggaccacgacaggcccgcagttatcaggtcatgaacggcatcgccgtgctgccggtgtccggcacgctggtcagccggacgcgggcgctgcagccgtactc

SEQ ID NO: 33 - DNA, 303 bp, Artificial Sequence
  Synthetic
  L9730-303
catttgaacataacggtgtgaccgtcacgctttctgaactgtcagccctgcagcgcattgagcatctcgccctgatgaaacggcaggcagaacaggcggagtcagacagcaaccggaagtttactgtggaagacgccatcagaaccggcgcgtttctggtggcgatgtccctgtggcataaccatccgcagaagacgcagatgccgtccatgaatgaagccgttaaacagattgagcaggaagtgcttaccacctggcccacggaggcaatttctcatgctgaaaacgtggtgtaccggctgt

SEQ ID NO: 34 - DNA, 301 bp, Artificial Sequence
  Synthetic
  L718-308
gtgttcgacggtgagctgagttttgccctgaaactggcgcgtgagatggggcgacccgactggcgtgccatgcttgccgggatgtcatccacggagtatgccgactggcaccgcttttacagtacccattattttcatgatgttctgctggatatgcacttttccgggctgacgtacaccgtgctcagcctgtttttcagcgatccggatatgcatccgctggatttcagtctgctgaaccggcgcgaggctgacgaagagcctgaagatgatgtgctgatgcagaaagcggcagggcttg

SEQ ID NO: 35 - DNA, 497 bp, Artificial Sequence
  Synthetic
  L29732-497
tactcaacccgatgtttgagtacggtcatcatctgacactacagactctggcatcgctgtgaagacgacgcgaaattcagcattttcacaagcgttatcttttacaaaaccgatctcactctcctttgatgcgaatgccagcgtcagacatcatatgcagatactcacctgcatcctgaacccattgacctccaaccccgtaatagcgatgcgtaatgatgtcgatagttactaacgggtcttgttcgattaactgccgcagaaactcttccaggtcaccagtgcagtgcttgataacaggagtcttcccaggatggcgaacaacaagaaactggtttccgtcttcacggacttcgttgctttccagtttagcaatacgcttactcccatccgagataacaccttcgtaatactcacgctgctcgttgagttttgattttgctgtttcaagctcaacacgcagtttccctactgttagcgcaatatcctcgttctcc

SEQ ID NO: 36 - DNA, 500 bp, Artificial Sequence
  Synthetic
  L501-500
actccgctgaagtggtggaaaccgcattctgtactttcgtgctgtcgcggatcgcaggtgaaattgccagtattctcgacgggctccccctgtcggtgcagcggcgttttccggaactggaaaaccgacatgttgatttcctgaaacgggatatcatcaaagccatgaacaaagcagccgcgctggatgaactgataccggggttgctgagtgaatatatcgaacagtcaggttaacaggctgcggcattttgtccgcgccgggcttcgctcactgttcaggccggagccacagaccgccgttgaatgggcggatgctaattactatctcccgaaagaatccgcataccaggaagggcgctgggaaacactgccctttcagcgggccatcatgaatgcgatgggcagcgactacatccgtgaggtgaatgtggtgaagtctgcccgtgtcggttattccaaaatgctgctgggtgtttatgcctactttatagagcataa

SEQ ID NO: 37 - DNA, 500 bp, Artificial Sequence
  Synthetic
  L30501-500
cactcacaacaatgagtggcagatatagcctggtggttcaggcggcgcatttttattgctgtgttgcgctgtaattcttctatttctgatgctgaatcaatgatgtctgccatctttcattaatccctgaactgttggttaatacgcttgagggtgaatgcgaataataaaaaaggagcctgtagctccctgatgattttgcttttcatgttcatcgttccttaaagacgccgtttaacatgccgattgccaggcttaaatgagtcggtgtgaatcccatcagcgttaccgtttcgcggtgcttcttcagtacgctacggcaaatgtcatcgacgtttttatccggaaactgctgtctggctttttttgatttcagaattagcctgacgggcaatgctgcgaagggcgttttcctgctgaggtgtcattgaacaagtcccatgtcggcaagcataagcacacagaatatgaagcccgctgccagaaaaatgcattccgtg

SEQ ID NO: 38 - DNA, 500 bp, Artificial Sequence
  Synthetic
  L46499-500
gcctaaagtaataaaaccgagcaatccatttacgaatgtttgctgggtttctgttttaacaacattttctgcgccgccacaaattttggctgcatcgacagttttcttctgcccaattccagaaacgaagaaatgatgggtgatggtttcctttggtgctactgctgccggtttgttttgaacagtaaacgtctgttgagcacatcctgtaataagcagggccagcgcagtagcgagtagcatttttttcatggtgttattcccgatgctttttgaagttcgcagaatcgtatgtgtagaaaattaaacaaaccctaaacaatgagttgaaatttcatattgttaatatttattaatgtatgtcaggtgcgatgaatcgtcattgtattcccggattaactatgtccacagccctgacggggaacttctctgcgggagtgtccgggaataattaaaacgatgcacacagggtttagcgcgtacacgtattgcattatgcc

SEQ ID NO: 39 - DNA, 1011 bp, Artificial Sequence
  Synthetic
  L8703-1012
aagagctggacagcgatacctggcaggcggagctgcatatcgaagttttcctgcctgctcaggtgccggattcagagctggatgcgtggatggagtcccggatttatccggtgatgagcgatatcccggcactgtcagatttgatcaccagtatggtggccagcggctatgactaccggcgcgacgatgatgcgggcttgtggagttcagccgatctgacttatgtcattacctatgaaatgtgaggacgctatgcctgtaccaaatcctacaatgccggtgaaaggtgccgggaccaccctgtgggtttataaggggagcggtgacccttacgcgaatccgctttcagacgttgactggtcgcgtctggcaaaagttaaagacctgacgcccggcgaactgaccgctgagtcctatgacgacagctatctcgatgatgaagatgcagactggactgcgaccgggcaggggcagaaatctgccggagataccagcttcacgctggcgtggatgcccggagagcaggggcagcaggcgctgctggcgtggtttaatgaaggcgatacccgtgcctataaaatccgcttcccgaacggcacggtcgatgtgttccgtggctgggtcagcagtatcggtaaggcggtgacggcgaaggaagtgatcacccgcacggtgaaagtcaccaatgtgggacgtccgtcgatggcagaagatcgcagcacggtaacagcggcaaccggcatgaccgtgacgcctgccagcacctcggtggtgaaagggcagagcaccacgctgaccgtggccttccagccggagggcgtaaccgacaagagctttcgtgcggtgtctgcggataaaacaaaagccaccgtgtcggtcagtggtatgaccatcaccgtgaacggcgttgctgcaggcaaggtcaacattccggttgtatccggtaatggtgagtttgctgcggttgcagaaattaccgtcaccgccagttaatccggagagtcagcgatg

SEQ ID NO: 40 - DNA, 32 bp, Artificial Sequence
  Synthetic
cctgtatgaccgtattccgggtcctgtcggta

SEQ ID NO: 41 - DNA, 425 bp, Artificial Sequence
  Synthetic
aagagctggacagcgatacctggcaggcggagctgcatatcgaagttttcctgcctgctcaggtgccggattcagagctggatgcgtggatggagtcccggatttatccggtgatgagcgatatcccggcactgtcagatttgatcaccagtatggtggccagcggctatgactaccggcgcgacgatgatgcgggcttgtggagttcagccgatctgacttatgtcattacctatgaaatgtgaggacgctatgcctgtaccaaatcctacaatgccggtgaaaggtgccgggaccaccctgtgggtttataaggggagcggtgacccttacgcgaatccgctttcagacgttgactggtcgcgtctggcaaaagttaaagacctgacgcccggcgaactgaccgctgagtcctatgacgacag